European Patent Application EP 4 599 857 A1, published August 13, 2025. Title: A Transdermal Photocuring Forming Hydrogel With Biological Activity As Well As A Preparation Method And An Application Thereof. Applicant: SHANXI JINBO BIO-PHARMACEUTICAL CO., LTD. Application US 18483493. The sequence listing filed with the application follows.

SEQUENCE LISTING (1 sequence)

SEQ ID NO: 1 - protein, 480 aa, recombinant collagen protein
GERGAPGFRGPAGPNGIPGEKGPAGERGAPGERGAPGFRGPAGPNGIPGEKGPAGERGAPGERGAPGFRGPAGPNGIPGEKGPAGERGAPGERGAPGFRGPAGPNGIPGEKGPAGERGAPGERGAPGFRGPAGPNGIPGEKGPAGERGAPGERGAPGFRGPAGPNGIPGEKGPAGERGAPGERGAPGFRGPAGPNGIPGEKGPAGERGAPGERGAPGFRGPAGPNGIPGEKGPAGERGAPGERGAPGFRGPAGPNGIPGEKGPAGERGAPGERGAPGFRGPAGPNGIPGEKGPAGERGAPGERGAPGFRGPAGPNGIPGEKGPAGERGAPGERGAPGFRGPAGPNGIPGEKGPAGERGAPGERGAPGFRGPAGPNGIPGEKGPAGERGAPGERGAPGFRGPAGPNGIPGEKGPAGERGAPGERGAPGFRGPAGPNGIPGEKGPAGERGAPGERGAPGFRGPAGPNGIPGEKGPAGERGAP